European Patent Application EP 4 223 772 A2, published August 9, 2023. Title: OPTIMIZED FACTOR VIII GENE. Applicant: Biogen MA Inc. Application EP. The sequence listing filed with the application follows.

SEQUENCE LISTING (51 sequences)

SEQ ID NO: 1 - DNA, 4404 bp, synthetic construct
  misc_feature 1..4404: note = optimized BDD FVIII
  source 1..4404: mol_type = other DNA
cgtacggccgccaccatgcagattgagctgtctacttgctttttcctgtgcctgctgaggttttgcttttccgctacacgaaggtattatctgggggctgtggaactgtcttgggattacatgcagagtgacctgggagagctgccagtggacgcaaggtttccccctagagtccctaagtcattccccttcaacactagcgtggtctacaagaaaacactgttcgtggagtttactgatcacctgttcaacatcgcaaagcctaggccaccctggatgggactgctggggccaacaatccaggccgaggtgtacgacaccgtggtcattacacttaagaacatggcctcacaccccgtgagcctgcatgctgtgggcgtcagctactggaaggcttccgaaggagcagagtatgacgatcagacttcccagagagaaaaagaggacgataaggtgtttcctggcggatctcatacctacgtgtggcaggtcctgaaagagaatggccctatggcctccgaccctctgtgcctgacctactcttatctgagtcacgtggacctggtcaaggatctgaacagcggcctgatcggagccctgctggtgtgcagggaaggaagcctggctaaggagaaaacccagacactgcataagttcattctgctgttcgccgtgtttgacgaagggaaatcatggcacagcgagacaaagaatagtctgatgcaggacagggatgccgcttcagccagagcttggcccaaaatgcacactgtgaacggctacgtcaatcgctcactgcctgggctgatcggctgccaccgaaagagcgtgtattggcatgtcatcgggatgggcaccacacctgaagtgcactccattttcctggagggacatacctttctggtccgcaaccaccgacaggcttccctggagatctctccaattaccttcctgacagcacagactctgctgatggacctggggcagttcctgctgttttgccacatcagctcccaccagcatgatggcatggaggcttacgtgaaagtggactcttgtcccgaggaacctcagctgcggatgaagaacaatgaggaagcagaagactatgacgatgacctgaccgactccgagatggatgtggtccgattcgatgacgataacagcccctcctttatccagattagatctgtggccaagaaacaccctaagacatgggtccattacatcgcagccgaggaagaggactgggattatgcaccactggtgctggcaccagacgatcgctcctacaaatctcagtatctgaacaatgggccacagaggattggcagaaagtacaagaaagtgcggttcatggcatataccgatgagaccttcaagactcgcgaagccatccagcacgagagcggcatcctgggaccactgctgtacggagaagtgggagacaccctgctgatcattttcaagaaccaggccagccggccttacaatatctatccacatgggattacagatgtgcgccctctgtacagcaggagactgccaaagggcgtcaaacacctgaaggacttcccaatcctgcccggagaaatcttcaagtacaagtggactgtcaccgtcgaggatggccccactaagagcgaccctcggtgcctgacccgctactattctagtttcgtgaatatggaaagagatctggcaagcggactgatcggaccactgctgatttgttacaaagagagcgtggatcagagaggcaaccagatcatgtccgacaagcggaatgtgattctgttcagtgtctttgacgaaaacaggtcatggtacctgaccgagaacatccagagattcctgcctaatccagctggggtgcagctggaagatcctgagtttcaggcatctaacatcatgcatagtattaatggctacgtgttcgacagtttgcagctgagcgtgtgcctgcacgaggtcgcttactggtatatcctgagcattggggcacagacagatttcctgagcgtgttcttttccggctacacttttaagcataaaatggtctatgaggacacactgactctgttccccttcagcggcgaaaccgtgtttatgagcatggagaatcccggactgtggattctggggtgccacaacagcgatttcagaaatcgcggaatgactgccctgctgaaagtgtcaagctgtgacaagaacaccggggactactatgaagattcatacgaggacatcagcgcatatctgctgtccaaaaacaatgccattgaaccccggtcttttagtcagaatcctccagtgctgaagcggcaccagcgcgagatcacccgcactaccctgcagagtgatcaggaagagatcgactacgacgatacaatttctgtggaaatgaagaaagaggacttcgatatctatgacgaagatgagaaccagagtcctcgatcattccagaagaaaaccaggcattactttattgccgcagtggagcggctgtgggattatggcatgtcctctagtcctcacgtgctgcgaaatagggcccagtcaggaagcgtcccacagttcaagaaagtggtcttccaggagtttacagacgggtcctttactcagccactgtacaggggcgaactgaacgagcacctgggactgctggggccctatatcagagcagaagtggaggataacattatggtcaccttcagaaatcaggcctctcggccttacagtttttattcaagcctgatctcttacgaagaggaccagcgacagggagctgaaccacgaaaaaacttcgtgaagcctaatgagaccaaaacatacttttggaaggtgcagcaccatatggccccaacaaaagacgagttcgattgcaaggcatgggcctatttttctgacgtggatctggagaaggacgtgcacagtggcctgattggcccactgctggtgtgccatactaacaccctgaatccagcccacggccggcaggtcactgtccaggagttcgctctgttctttaccatctttgatgagacaaagagctggtacttcaccgaaaacatggagcgaaattgcagggctccatgtaacattcagatggaagaccccacattcaaggagaactaccgctttcatgctatcaatggatacatcatggatactctgcccgggctggtcatggcacaggaccagagaatccggtggtatctgctgagcatgggcagcaacgagaatatccactcaattcatttcagcgggcacgtgtttactgtcaggaagaaagaagagtacaagatggccctgtacaacctgtatcccggcgtgttcgaaaccgtcgagatgctgcctagcaaggccggaatctggagagtggaatgcctgattggagagcacctgcatgctgggatgtctaccctgtttctggtgtacagtaataagtgtcagacacccctgggaatggcatccgggcatatcagggatttccagattaccgcatctggacagtacggacagtgggcacctaagctggctagactgcactattccggatctatcaacgcttggtccacaaaagagcctttctcttggattaaggtggacctgctggccccaatgatcattcatggcatcaaaactcagggagctcggcagaagttctcctctctgtacatctcacagtttatcatcatgtacagcctggatgggaagaaatggcagacataccgcggcaatagcacaggaactctgatggtgttctttggcaacgtggacagcagcggaatcaagcacaacattttcaatccccctatcattgctagatacatccggctgcacccaacccattattctattcgaagtacactgaggatggaactgatgggatgcgatctgaacagttgttcaatgcccctggggatggagtccaaggcaatctctgacgcccagattaccgctagctcctacttcactaatatgtttgctacctggagcccttccaaagcaagactgcacctgcaaggccgcagcaacgcatggcgaccacaggtgaacaatcccaaggagtggttgcaggtcgattttcagaaaactatgaaggtgaccggggtcacaactcagggcgtgaaaagtctgctgacctcaatgtacgtcaaggagttcctgatctctagttcacaggacggacatcagtggacactgttctttcagaacgggaaggtgaaagtcttccagggcaatcaggattcctttacacctgtggtcaacagtctagaccctccactgctgaccagatacctgagaatccaccctcagtcctgggtgcaccagattgccctgagaatggaagtgctgggatgcgaggcccaggatctgtactgataactcgagtcgacc

SEQ ID NO: 2 - DNA, 4419 bp, synthetic construct
  misc_feature 1..4419: note = optimized BDD FVIII
  source 1..4419: mol_type = other DNA
ggcgcgcccgtacggccgccaccatgcagatcgagctgtctacctgcttcttcctgtgcctgctgcggttctgcttcagcgccacccggcggtactacctgggcgccgtggaactgagctgggactacatgcagagcgacctgggggagctgcccgtggacgccagattccccccaagagtgcccaagagcttccccttcaacacctccgtggtgtacaagaaaaccctgttcgtcgagttcaccgaccacctgttcaatatcgccaagcccagacccccctggatgggcctgctgggccctacaatccaggccgaggtgtacgacaccgtggtcatcacccttaagaacatggccagccaccccgtgtccctgcacgccgtgggcgtgtcctactggaaggcctctgagggcgctgagtacgacgaccagaccagccagcgcgagaaagaggacgacaaagtctttcctggcggcagccatacctacgtgtggcaggtcctgaaagaaaacggccctatggcctccgaccccctgtgcctgacctacagctacctgagccacgtggacctggtcaaggacctgaacagcggcctgattggcgccctgctcgtgtgtagagagggcagcctcgccaaagagaaaacccagaccctgcacaagttcatcctgctgttcgccgtgttcgacgagggcaagagctggcacagcgagacaaagaacagcctgatgcaggaccgggacgccgcctctgccagagcctggcctaagatgcacaccgtgaacggctacgtgaacagaagcctgcccggactgatcggctgccaccggaagtccgtgtactggcacgtgatcggcatgggcaccacccccgaggtgcacagcatctttctggaaggccacaccttcctcgtgcggaaccacagacaggccagcctggaaatcagccctatcaccttcctgaccgcccagacactgctgatggacctgggccagttcctgctgttttgccacatcagcagccaccagcacgacggcatggaagcctacgtgaaggtggacagctgccccgaggaaccccagctgcggatgaagaacaacgaggaagccgaggactacgacgacgacctgaccgacagcgagatggacgtcgtgcgcttcgacgacgacaacagccccagcttcatccagatcagaagcgtggccaagaagcaccccaagacctgggtgcactatatcgccgccgaggaagaggactgggactacgcccctctggtgctggcccccgacgacagaagctacaagagccagtacctgaacaatggcccccagcggatcggccggaagtacaagaaagtgcggttcatggcctacaccgacgagacattcaagaccagagaggccatccagcacgagagcggcatcctgggccccctgctgtatggcgaagtgggcgacaccctgctgatcatcttcaagaaccaggccagccggccctacaacatctacccccacggcatcaccgacgtgcggcccctgtacagcagacggctgcccaagggcgtgaagcacctgaaggacttccccatcctgcccggcgagatcttcaagtacaagtggaccgtgaccgtggaagatggccccaccaagagcgaccccagatgcctgacccggtactacagcagcttcgtgaacatggaacgggacctggcctccgggctgatcggccctctgctgatctgctacaaagaaagcgtggaccagcggggcaaccagatcatgagcgacaagcggaacgtgatcctgttcagcgtgttcgatgagaatcggtcctggtacctgaccgagaatatccagcggttcctgcccaaccctgccggcgtgcagctggaagatcccgagttccaggccagcaacatcatgcactccatcaatggctacgtgttcgacagcctccagctgagcgtgtgcctgcacgaggtggcctactggtacatcctgagcatcggcgcccagaccgacttcctgagcgtgttcttcagcggctacaccttcaagcacaagatggtgtacgaggataccctgaccctgttccccttctccggcgaaaccgtgttcatgagcatggaaaaccccggcctgtggattctgggctgccacaacagcgacttcagaaaccggggcatgaccgccctgctgaaggtgtccagctgcgacaagaacaccggcgactactacgaggacagctatgaggacatcagcgcctacctgctgagcaagaacaacgccatcgagcccagatccttcagccagaacccccccgtgctgaagcggcaccagagagagatcacccggaccaccctgcagtccgaccaggaagagattgattacgacgacaccatcagcgtcgagatgaagaaagaggatttcgacatctacgacgaggacgagaaccagagcccccggtccttccagaagaaaacccggcactacttcattgccgccgtggaaagactgtgggactacggcatgagcagcagcccccacgtgctgcggaacagagcccagagcggcagcgtgccccagttcaagaaagtggtgttccaggagttcaccgacggcagcttcacccagcccctgtatcggggcgagctgaacgagcacctgggactgctgggaccttacattagagccgaggtggaagataacatcatggtcaccttcagaaaccaggcctccagaccctacagcttctacagcagcctgatcagctacgaagaggaccagcggcagggcgccgaaccccggaagaacttcgtgaagcccaacgagactaagacctacttctggaaggtgcagcaccacatggcccccacaaaggacgagttcgactgcaaggcctgggcctacttctccgatgtggacctggaaaaggacgtgcactctggcctgattggacctctgctcgtctgccacaccaacaccctgaaccccgcccacggccggcaggtcacagtgcaggaatttgccctgttcttcaccatcttcgatgagacaaagagctggtacttcaccgagaacatggaaagaaactgtagagccccctgcaacatccagatggaagatcctaccttcaaagagaactatcggttccacgccatcaacggctacatcatggacaccctgcccggcctggtcatggcccaggatcagagaatccggtggtatctgctgagcatgggcagcaacgagaacatccacagcatccacttcagcggccacgtgttcacagtgcggaagaaagaagagtacaagatggccctgtacaacctgtaccccggcgtgttcgagacagtggaaatgctgcccagcaaggccggcatctggcgggtggaatgtctgatcggcgagcatctgcacgccggaatgagcaccctgtttctggtgtacagcaacaagtgccagacccctctgggcatggccagcggccacatccgggacttccagatcaccgcctccggccagtacggccagtgggcccctaagctggcccggctccactactccggatctatcaacgcctggtccaccaaagagcccttcagctggatcaaggtggacctgctggcccctatgatcatccacggaatcaagacccagggcgccagacagaagttcagcagcctgtacatcagccagttcatcatcatgtacagcctggacggcaagaagtggcagacctaccggggcaacagcaccggcaccctgatggtgttcttcggcaacgtggacagcagcggcatcaagcacaacatcttcaacccccccatcattgcccggtacatccggctgcaccccacccactacagcatccggtccaccctgcggatggaactgatgggctgcgacctgaactcttgcagcatgcccctggggatggaaagcaaggccatcagcgacgcccagatcacagccagcagctacttcaccaacatgttcgccacctggtccccaagcaaagcccgcctgcatctccaaggcagaagcaatgcctggcggcctcaggtcaacaaccccaaagaatggctccaggtggactttcagaaaaccatgaaggtcacaggcgtgaccacccagggcgtgaaaagcctgctgacctctatgtacgtgaaagagttcctgatcagcagcagccaggacgggcaccagtggaccctgttctttcagaacggcaaagtgaaagtgttccagggcaaccaggactcctttacccccgtggtcaactctctagaccctccactgctgaccagatacctgagaatccaccctcagtcctgggtgcaccagattgccctgagaatggaagtgctgggatgcgaggcccaggatctgtactgataactcgagtcgacttaattaa

SEQ ID NO: 3 - DNA, 4371 bp, synthetic construct
  misc_feature 1..4371: note = Parental BDD FVIII
  source 1..4371: mol_type = other DNA
atgcaaatagagctctccacctgcttctttctgtgccttttgcgattctgctttagtgccaccagaagatactacctgggtgcagtggaactgtcatgggactatatgcaaagtgatctcggtgagctgcctgtggacgcaagatttcctcctagagtgccaaaatcttttccattcaacacctcagtcgtgtacaaaaagactctgtttgtagaattcacggatcaccttttcaacatcgctaagccaaggccaccctggatgggtctgctaggtcctaccatccaggctgaggtttatgatacagtggtcattacacttaagaacatggcttcccatcctgtcagtcttcatgctgttggtgtatcctactggaaagcttctgagggagctgaatatgatgatcagaccagtcaaagggagaaagaagatgataaagtcttccctggtggaagccatacatatgtctggcaggtcctgaaagagaatggtccaatggcctctgacccactgtgccttacctactcatatctttctcatgtggacctggtaaaagacttgaattcaggcctcattggagccctactagtatgtagagaagggagtctggccaaggaaaagacacagaccttgcacaaatttatactactttttgctgtatttgatgaagggaaaagttggcactcagaaacaaagaactccttgatgcaggatagggatgctgcatctgctcgggcctggcctaaaatgcacacagtcaatggttatgtaaacaggtctctgccaggtctgattggatgccacaggaaatcagtctattggcatgtgattggaatgggcaccactcctgaagtgcactcaatattcctcgaaggtcacacatttcttgtgaggaaccatcgccaggcgtccttggaaatctcgccaataactttccttactgctcaaacactcttgatggaccttggacagtttctactgttttgtcatatctcttcccaccaacatgatggcatggaagcttatgtcaaagtagacagctgtccagaggaaccccaactacgaatgaaaaataatgaagaagcggaagactatgatgatgatcttactgattctgaaatggatgtggtcaggtttgatgatgacaactctccttcctttatccaaattcgctcagttgccaagaagcatcctaaaacttgggtacattacattgctgctgaagaggaggactgggactatgctcccttagtcctcgcccccgatgacagaagttataaaagtcaatatttgaacaatggccctcagcggattggtaggaagtacaaaaaagtccgatttatggcatacacagatgaaacctttaagactcgtgaagctattcagcatgaatcaggaatcttgggacctttactttatggggaagttggagacacactgttgattatatttaagaatcaagcaagcagaccatataacatctaccctcacggaatcactgatgtccgtcctttgtattcaaggagattaccaaaaggtgtaaaacatttgaaggattttccaattctgccaggagaaatattcaaatataaatggacagtgactgtagaagatgggccaactaaatcagatcctcggtgcctgacccgctattactctagtttcgttaatatggagagagatctagcttcaggactcattggccctctcctcatctgctacaaagaatctgtagatcaaagaggaaaccagataatgtcagacaagaggaatgtcatcctgttttctgtatttgatgagaaccgaagctggtacctcacagagaatatacaacgctttctccccaatccagctggagtgcagcttgaggatccagagttccaagcctccaacatcatgcacagcatcaatggctatgtttttgatagtttgcagttgtcagtttgtttgcatgaggtggcatactggtacattctaagcattggagcacagactgacttcctttctgtcttcttctctggatataccttcaaacacaaaatggtctatgaagacacactcaccctattcccattctcaggagaaactgtcttcatgtcgatggaaaacccaggtctatggattctggggtgccacaactcagactttcggaacagaggcatgaccgccttactgaaggtttctagttgtgacaagaacactggtgattattacgaggacagttatgaagatatttcagcatacttgctgagtaaaaacaatgccattgaaccaagaagcttctctcaaaacccaccagtcttgaaacgccatcaacgggaaataactcgtactactcttcagtcagatcaagaggaaattgactatgatgataccatatcagttgaaatgaagaaggaagattttgacatttatgatgaggatgaaaatcagagcccccgcagctttcaaaagaaaacacgacactattttattgctgcagtggagaggctctgggattatgggatgagtagctccccacatgttctaagaaacagggctcagagtggcagtgtccctcagttcaagaaagttgttttccaggaatttactgatggctcctttactcagcccttataccgtggagaactaaatgaacatttgggactcctggggccatatataagagcagaagttgaagataatatcatggtaactttcagaaatcaggcctctcgtccctattccttctattctagccttatttcttatgaggaagatcagaggcaaggagcagaacctagaaaaaactttgtcaagcctaatgaaaccaaaacttacttttggaaagtgcaacatcatatggcacccactaaagatgagtttgactgcaaagcctgggcttatttctctgatgttgacctggaaaaagatgtgcactcaggcctgattggaccccttctggtctgccacactaacacactgaaccctgctcatgggagacaagtgacagtacaggaatttgctctgtttttcaccatctttgatgagaccaaaagctggtacttcactgaaaatatggaaagaaactgcagggctccctgcaatatccagatggaagatcccacttttaaagagaattatcgcttccatgcaatcaatggctacataatggatacactacctggcttagtaatggctcaggatcaaaggattcgatggtatctgctcagcatgggcagcaatgaaaacatccattctattcatttcagtggacatgtgttcactgtacgaaaaaaagaggagtataaaatggcactgtacaatctctatccaggtgtttttgagacagtggaaatgttaccatccaaagctggaatttggcgggtggaatgccttattggcgagcatctacatgctgggatgagcacactttttctggtgtacagcaataagtgtcagactcccctgggaatggcttctggacacattagagattttcagattacagcttcaggacaatatggacagtgggccccaaagctggccagacttcattattccggatcaatcaatgcctggagcaccaaggagcccttttcttggatcaaggtggatctgttggcaccaatgattattcacggcatcaagacccagggtgcccgtcagaagttctccagcctctacatctctcagtttatcatcatgtatagtcttgatgggaagaagtggcagacttatcgaggaaattccactggaaccttaatggtcttctttggcaatgtggattcatctgggataaaacacaatatttttaaccctccaattattgctcgatacatccgtttgcacccaactcattatagcattcgcagcactcttcgcatggagttgatgggctgtgatttaaatagttgcagcatgccattgggaatggagagtaaagcaatatcagatgcacagattactgcttcatcctactttaccaatatgtttgccacctggtctccttcaaaagctcgacttcacctccaagggaggagtaatgcctggagacctcaggtgaataatccaaaagagtggctgcaagtggacttccagaagacaatgaaagtcacaggagtaactactcagggagtaaaatctctgcttaccagcatgtatgtgaaggagttcctcatctccagcagtcaagatggccatcagtggactctcttttttcagaatggcaaagtaaaggtttttcagggaaatcaagactccttcacacctgtggtgaactctctagacccaccgttactgactcgctaccttcgaattcacccccagagttgggtgcaccagattgccctgaggatggaggttctgggctgcgaggcacaggacctctac

SEQ ID NO: 4 - protein, 1438 aa, synthetic construct
  REGION 1..1438: note = BDD FVIII
ATRRYYLGAVELSWDYMQSDLGELPVDARFPPRVPKSFPFNTSVVYKKTLFVEFTDHLFNIAKPRPPWMGLLGPTIQAEVYDTVVITLKNMASHPVSLHAVGVSYWKASEGAEYDDQTSQREKEDDKVFPGGSHTYVWQVLKENGPMASDPLCLTYSYLSHVDLVKDLNSGLIGALLVCREGSLAKEKTQTLHKFILLFAVFDEGKSWHSETKNSLMQDRDAASARAWPKMHTVNGYVNRSLPGLIGCHRKSVYWHVIGMGTTPEVHSIFLEGHTFLVRNHRQASLEISPITFLTAQTLLMDLGQFLLFCHISSHQHDGMEAYVKVDSCPEEPQLRMKNNEEAEDYDDDLTDSEMDVVRFDDDNSPSFIQIRSVAKKHPKTWVHYIAAEEEDWDYAPLVLAPDDRSYKSQYLNNGPQRIGRKYKKVRFMAYTDETFKTREAIQHESGILGPLLYGEVGDTLLIIFKNQASRPYNIYPHGITDVRPLYSRRLPKGVKHLKDFPILPGEIFKYKWTVTVEDGPTKSDPRCLTRYYSSFVNMERDLASGLIGPLLICYKESVDQRGNQIMSDKRNVILFSVFDENRSWYLTENIQRFLPNPAGVQLEDPEFQASNIMHSINGYVFDSLQLSVCLHEVAYWYILSIGAQTDFLSVFFSGYTFKHKMVYEDTLTLFPFSGETVFMSMENPGLWILGCHNSDFRNRGMTALLKVSSCDKNTGDYYEDSYEDISAYLLSKNNAIEPRSFSQNPPVLKRHQREITRTTLQSDQEEIDYDDTISVEMKKEDFDIYDEDENQSPRSFQKKTRHYFIAAVERLWDYGMSSSPHVLRNRAQSGSVPQFKKVVFQEFTDGSFTQPLYRGELNEHLGLLGPYIRAEVEDNIMVTFRNQASRPYSFYSSLISYEEDQRQGAEPRKNFVKPNETKTYFWKVQHHMAPTKDEFDCKAWAYFSDVDLEKDVHSGLIGPLLVCHTNTLNPAHGRQVTVQEFALFFTIFDETKSWYFTENMERNCRAPCNIQMEDPTFKENYRFHAINGYIMDTLPGLVMAQDQRIRWYLLSMGSNENIHSIHFSGHVFTVRKKEEYKMALYNLYPGVFETVEMLPSKAGIWRVECLIGEHLHAGMSTLFLVYSNKCQTPLGMASGHIRDFQITASGQYGQWAPKLARLHYSGSINAWSTKEPFSWIKVDLLAPMIIHGIKTQGARQKFSSLYISQFIIMYSLDGKKWQTYRGNSTGTLMVFFGNVDSSGIKHNIFNPPIIARYIRLHPTHYSIRSTLRMELMGCDLNSCSMPLGMESKAISDAQITASSYFTNMFATWSPSKARLHLQGRSNAWRPQVNNPKEWLQVDFQKTMKVTGVTTQGVKSLLTSMYVKEFLISSSQDGHQWTLFFQNGKVKVFQGNQDSFTPVVNSLDPPLLTRYLRIHPQSWVHQIALRMEVLGCEAQDLY

SEQ ID NO: 5-15 - skipped (11 entries)

SEQ ID NO: 16 - DNA, 13 bp, synthetic construct
  misc_feature 1..13: note = Kozak Consensus Sequence
  source 1..13: mol_type = other DNA
gccgccaccatgc

SEQ ID NO: 17 - protein, 32 aa, synthetic construct
  REGION 1..32: note = CTP peptide
DPRFQDSSSSKAPPPSLPSPSRLPGPSDTPIL

SEQ ID NO: 18 - protein, 28 aa, synthetic construct
  REGION 1..28: note = CTP peptide
SSSSKAPPPSLPSPSRLPGPSDTPILPQ

SEQ ID NO: 19 - protein, 11 aa, synthetic construct
  REGION 1..11: note = albumin-binding peptides core sequence
DICLPRWGCLW

SEQ ID NO: 20 - protein, 20 aa, synthetic construct
  REGION 1..20: note = PAS Sequence
ASPAAPAPASPAAPAPSAPA

SEQ ID NO: 21 - protein, 20 aa, synthetic construct
  REGION 1..20: note = PAS Sequence
AAPASPAPAAPSAPAPAAPS

SEQ ID NO: 22 - protein, 20 aa, synthetic construct
  REGION 1..20: note = PAS Sequence
APSSPSPSAPSSPSPASPSS

SEQ ID NO: 23 - protein, 19 aa, synthetic construct
  REGION 1..19: note = PAS Sequence
APSSPSPSAPSSPSPASPS

SEQ ID NO: 24 - protein, 20 aa, synthetic construct
  REGION 1..20: note = PAS Sequence
SSPSAPSPSSPASPSPSSPA

SEQ ID NO: 25 - protein, 24 aa, synthetic construct
  REGION 1..24: note = PAS Sequence
AASPAAPSAPPAAASPAAPSAPPA

SEQ ID NO: 26 - protein, 20 aa, synthetic construct
  REGION 1..20: note = PAS Sequence
ASAAAPAAASAAASAPSAAA

SEQ ID NO: 27 - DNA, 16842 bp, Homo sapiens
  source 1..16842: mol_type = other DNA
atgattcctgccagatttgccggggtgctgcttgctctggccctcattttgccagggaccctttgtgcagaaggaactcgcggcaggtcatccacggccctactaaggacggtctaaacggccccacgacgaacgagaccgggagtaaaacggtccctgggaaacacgtcttccttgagcgccgtccagtaggtgccggggatgcagccttttcggaagtgacttcgtcaacacctttgatgggagcatgtacagctttgcgggatactgcagttacctcctggcagggggctgccagaactacgtcggaaaagccttcactgaagcagttgtggaaactaccctcgtacatgtcgaaacgccctatgacgtcaatggaggaccgtcccccgacggtcttacgctccttctcgattattggggacttccagaatggcaagagagtgagcctctccgtgtatcttggggaattttttgacatccatttgtttgtcaatggttgcgaggaagagctaataacccctgaaggtcttaccgttctctcactcggagaggcacatagaaccccttaaaaaactgtaggtaaacaaacagttaccaaccgtgacacagggggaccaaagagtctccatgccctatgcctccaaagggctgtatctagaaactgaggctgggtactacaagctgtccggtgaggccttggcactgtgtccccctggtttctcagaggtacgggatacggaggtttcccgacatagatctttgactccgacccatgatgttcgacaggccactccggaatggctttgtggccaggatcgatggcagcggcaactttcaagtcctgctgtcagacagatacttcaacaagacctgcgggctgtgtggcaactttaacattaccgaaacaccggtcctagctaccgtcgccgttgaaagttcaggacgacagtctgtctatgaagttgttctggacgcccgacacaccgttgaaattgtactttgctgaagatgactttatgacccaagaagggaccttgacctcggacccttatgactttgccaactcatgggctctgagcagtggagaacagtggtgtgaaacgacttctactgaaatactgggttcttccctggaactggagcctgggaatactgaaacggttgagtacccgagactcgtcacctcttgtcaccacagaacgggcatctcctcccagcagctcatgcaacatctcctctggggaaatgcagaagggcctgtgggagcagtgccagcttctgaagagcacctcggtgtcttgcccgtagaggagggtcgtcgagtacgttgtagaggagacccctttacgtcttcccggacaccctcgtcacggtcgaagacttctcgtggagccacattgcccgctgccaccctctggtggaccccgagccttttgtggccctgtgtgagaagactttgtgtgagtgtgctggggggctggagtgcgcctgccctgcaacgggcgacggtgggagaccacctggggctcggaaaacaccgggacacactcttctgaaacacactcacacgaccccccgacctcacgcggacgggacgcctcctggagtacgcccggacctgtgcccaggagggaatggtgctgtacggctggaccgaccacagcgcgtgcagcccagtgtgccctgctggtatggagggaggacctcatgcgggcctggacacgggtcctcccttaccacgacatgccgacctggctggtgtcgcgcacgtcgggtcacacgggacgaccatacctctataggcagtgtgtgtccccttgcgccaggacctgccagagcctgcacatcaatgaaatgtgtcaggagcgatgcgtggatggctgcagctgccctgaggatatccgtcacacacaggggaacgcggtcctggacggtctcggacgtgtagttactttacacagtcctcgctacgcacctaccgacgtcgacgggactccgacagctcctggatgaaggcctctgcgtggagagcaccgagtgtccctgcgtgcattccggaaagcgctaccctcccggcacctccctctctcgagactgctgtcgaggacctacttccggagacgcacctctcgtggctcacagggacgcacgtaaggcctttcgcgatgggagggccgtggagggagagagctctgaccaacacctgcatttgccgaaacagccagtggatctgcagcaatgaagaatgtccaggggagtgccttgtcactggtcaatcccacttcaagagctttgacgttgtggacgtaaacggctttgtcggtcacctagacgtcgttacttcttacaggtcccctcacggaacagtgaccagttagggtgaagttctcgaaactgaacagatacttcaccttcagtgggatctgccagtacctgctggcccgggattgccaggaccactccttctccattgtcattgagactgtccagtgtgctgttgtctatgaagtggaagtcaccctagacggtcatggacgaccgggccctaacggtcctggtgaggaagaggtaacagtaactctgacaggtcacacgacatgaccgcgacgctgtgtgcacccgctccgtcaccgtccggctgcctggcctgcacaacagccttgtgaaactgaagcatggggcaggagttgccatggatactggcgctgcgacacacgtgggcgaggcagtggcaggccgacggaccggacgtgttgtcggaacactttgacttcgtaccccgtcctcaacggtaccttggccaggacatccagctccccctcctgaaaggtgacctccgcatccagcatacagtgacggcctccgtgcgcctcagctacggggaggacctgcagatgaccggtcctgtaggtcgagggggaggactttccactggaggcgtaggtcgtatgtcactgccggaggcacgcggagtcgatgcccctcctggacgtctacgactgggatggccgcgggaggctgctggtgaagctgtcccccgtctatgccgggaagacctgcggcctgtgtgggaattacaatggcaaccagggcgacgctgaccctaccggcgccctccgacgaccacttcgacagggggcagatacggcccttctggacgccggacacacccttaatgttaccgttggtcccgctgcacttccttaccccctctgggctggcrgagccccgggtggaggacttcgggaacgcctggaagctgcacggggactgccaggacctgcagaagcagcacagtgaaggaatgggggagacccgaccgyctcggggcccacctcctgaagcccttgcggaccttcgacgtgcccctgacggtcctggacgtcttcgtcgtgtccgatccctgcgccctcaacccgcgcatgaccaggttctccgaggaggcgtgcgcggtcctgacgtcccccacattcgaggcctgccatcgtgccgtcagcgctagggacgcgggagttgggcgcgtactggtccaagaggctcctccgcacgcgccaggactgcagggggtgtaagctccggacggtagcacggcagtcgccgctgccctacctgcggaactgccgctacgacgtgtgctcctgctcggacggccgcgagtgcctgtgcggcgccctggccagctatgccgcggcctgcgggcgacgggatggacgccttgacggcgatgctgcacacgaggacgagcctgccggcgctcacggacacgccgcgggaccggtcgatacggcgccggacgccggggagaggcgtgcgcgtcgcgtggcgcgagccaggccgctgtgagctgaactgcccgaaaggccaggtgtacctgcagtgcgggaccccctgcaacctgcccctctccgcacgcgcagcgcaccgcgctcggtccggcgacactcgacttgacgggctttccggtccacatggacgtcacgccctgggggacgttggagacctgccgctctctctcttacccggatgaggaatgcaatgaggcctgcctggagggctgcttctgccccccagggctctacatggatgagaggggggacctggacggcgagagagagaatgggcctactccttacgttactccggacggacctcccgacgaagacggggggtcccgagatgtacctactctcccccctgtgcgtgcccaaggcccagtgcccctgttactatgacggtgagatcttccagccagaagacatcttctcagaccatcacaccatgtgctactgtgaggatgacgcacgggttccgggtcacggggacaatgatactgccactctagaaggtcggtcttctgtagaagagtctggtagtgtggtacacgatgacactcctacgcttcatgcactgtaccatgagtggagtccccggaagcttgctgcctgacgctgtcctcagcagtcccctgtctcatcgcagcaaaaggagcctatcctgcgaagtacgtgacatggtactcacctcaggggccttcgaacgacggactgcgacaggagtcgtcaggggacagagtagcgtcgttttcctcggataggactcggccccccatggtcaagctggtgtgtcccgctgacaacctgcgggctgaagggctcgagtgtaccaaaacgtgccagaactatgacctggagtgcatgagccggggggtaccagttcgaccacacagggcgactgttggacgcccgacttcccgagctcacatggttttgcacggtcttgatactggacctcacgtacagcatgggctgtgtctctggctgcctctgccccccgggcatggtccggcatgagaacagatgtgtggccctggaaaggtgtccctgcttccatcagggcatcgtacccgacacagagaccgacggagacggggggcccgtaccaggccgtactcttgtctacacaccgggacctttccacagggacgaaggtagtcccgtaggagtatgcccctggagaaacagtgaagattggctgcaacacttgtgtctgtcgggaccggaagtggaactgcacagaccatgtgtgtgatgccacgtgtcctcatacggggacctctttgtcacttctaaccgacgttgtgaacacagacagccctggccttcaccttgacgtgtctggtacacacactacggtgcacctccacgatcggcatggcccactacctcaccttcgacgggctcaaatacctgttccccggggagtgccagtacgttctggtgcaggattactgcggcagtgaggtgctagccgtaccgggtgatggagtggaagctgcccgagtttatggacaaggggcccctcacggtcatgcaagaccacgtcctaatgacgccgtcaaaccctgggacctttcggatcctagtggggaataagggatgcagccacccctcagtgaaatgcaagaaacgggtcaccatcctggtggagggaggagagattgggaccctggaaagcctaggatcaccccttattccctacgtcggtggggagtcactttacgttctttgcccagtggtaggaccacctccctcctctctttgagctgtttgacggggaggtgaatgtgaagaggcccatgaaggatgagactcactttgaggtggtggagtctggccggtacatcattctgctgctgggaactcgacaaactgcccctccacttacacttctccgggtacttcctactctgagtgaaactccaccacctcagaccggccatgtagtaagacgacgaccccaaagccctctccgtggtctgggaccgccacctgagcatctccgtggtcctgaagcagacataccaggagaaagtgtgtggcctgtgtgggaattttgatgtttcgggagaggcaccagaccctggcggtggactcgtagaggcaccaggacttcgtctgtatggtcctctttcacacaccggacacacccttaaaactaggcatccagaacaatgacctcaccagcagcaacctccaagtggaggaagaccctgtggactttgggaactcctggaaagtgagctcgcagtgtgctgacaccgtaggtcttgttactggagtggtcgtcgttggaggttcacctccttctgggacacctgaaacccttgaggacctttcactcgagcgtcacacgactgtccagaaaagtgcctctggactcatcccctgccacctgccataacaacatcatgaagcagacgatggtggattcctcctgtagaatccttaccagtgacgtggtcttttcacggagacctgagtaggggacggtggacggtattgttgtagtacttcgtctgctaccacctaaggaggacatcttaggaatggtcactgcacttccaggactgcaacaagctggtggaccccgagccatatctggatgtctgcatttacgacacctgctcctgtgagtccattggggactgcgcctgcttcgaaggtcctgacgttgttcgaccacctggggctcggtatagacctacagacgtaaatgctgtggacgaggacactcaggtaacccctgacgcggacgaagtgcgacaccattgctgcctatgcccacgtgtgtgcccagcatggcaaggtggtgacctggaggacggccacattgtgcccccagagctgcgaggagaggaacgctgtggtaacgacggatacgggtgcacacacgggtcgtaccgttccaccactggacctcctgccggtgtaacacgggggtctcgacgctcctctcctatctccgggagaacgggtatgagtgtgagtggcgctataacagctgtgcacctgcctgtcaagtcacgtgtcagcaccctgagccactggcctgccctgttagaggccctcttgcccatactcacactcaccgcgatattgtcgacacgtggacggacagttcagtgcacagtcgtgggactcggtgaccggacgggacagcagtgtgtggagggctgccatgcccactgccctccagggaaaatcctggatgagcttttgcagacctgcgttgaccctgaagactgtccagtgtgtgagcgtcacacacctcccgacggtacgggtgacgggaggtcccttttaggacctactcgaaaacgtctggacgcaactgggacttctgacaggtcacacactcgtggctggccggcgttttgcctcaggaaagaaagtcaccttgaatcccagtgaccctgagcactgccagatttgccactgtgatgttgtcaacctcacctcaccgaccggccgcaaaacggagtcctttctttcagtggaacttagggtcactgggactcgtgacggtctaaacggtgacactacaacagttggagtggagtgaagcctgccaggagccgggaggcctggtggtgcctcccacagatgccccggtgagccccaccactctgtatgtggaggacatctcggaaccgccgttcacttcggacggtcctcggccctccggaccaccacggagggtgtctacggggccactcggggtggtgagacatacacctcctgtagagccttggcggcaagcacgatttctactgcagcaggctactggacctggtcttcctgctggatggctcctccaggctgtccgaggctgagtttgaagtgctgaaggcctttgtgcgtgctaaagatgacgtcgtccgatgacctggaccagaaggacgacctaccgaggaggtccgacaggctccgactcaaacttcacgacttccggaaacacgtggacatgatggagcggctgcgcatctcccagaagtgggtccgcgtggccgtggtggagtaccacgacggctcccacgcctacatcgggctcaaggacccacctgtactacctcgccgacgcgtagagggtcttcacccaggcgcaccggcaccacctcatggtgctgccgagggtgcggatgtagcccgagttcctggggaagcgaccgtcagagctgcggcgcattgccagccaggtgaagtatgcgggcagccaggtggcctccaccagcgaggtcttgaaatacacactgttccaccttcgctggcagtctcgacgccgcgtaacggtcggtccacttcatacgcccgtcggtccaccggaggtggtcgctccagaactttatgtgtgacaaggtaatcttcagcaagatcgaccgccctgaagcctcccgcatcgccctgctcctgatggccagccaggagccccaacggatgtcccggaactttgtccgctacttagaagtcgttctagctggcgggacttcggagggcgtagcgggacgaggactaccggtcggtcctcggggttgcctacagggccttgaaacaggcgatggtccagggcctgaagaagaagaaggtcattgtgatcccggtgggcattgggccccatgccaacctcaagcagatccgcctcatcgagaagcaggcccctgcaggtcccggacttcttcttcttccagtaacactagggccacccgtaacccggggtacggttggagttcgtctaggcggagtagctcttcgtccggggacagaacaaggccttcgtgctgagcagtgtggatgagctggagcagcaaagggacgagatcgttagctacctctgtgaccttgcccctgaagcccctcctcctcttgttccggaagcacgactcgtcacacctactcgacctcgtcgtttccctgctctagcaatcgatggagacactggaacggggacttcggggaggaggtactctgccccccgacatggcacaagtcactgtgggcccggggctcttgggggtttcgaccctggggcccaagaggaactccatggttctggatgtggcgatgagacggggggctgtaccgtgttcagtgacacccgggccccgagaacccccaaagctgggaccccgggttctccttgaggtaccaagacctacaccgcttcgtcctggaaggatcggacaaaattggtgaagccgacttcaacaggagcaaggagttcatggaggaggtgattcagcggatggatgtgggccaggacaaagcaggaccttcctagcctgttttaaccacttcggctgaagttgtcctcgttcctcaagtacctcctccactaagtcgcctacctacacccggtcctgtgcatccacgtcacggtgctgcagtactcctacatggtgaccgtggagtaccccttcagcgaggcacagtccaaaggggacatcctgcagcgggtgcgagacgtaggtgcagtgccacgacgtcatgaggatgtaccactggcacctcatggggaagtcgctccgtgtcaggtttcccctgtaggacgtcgcccacgctctgatccgctaccagggcggcaacaggaccaacactgggctggccctgcggtacctctctgaccacagcttcttggtcagccagggtgaccgggagcaggcgctaggcgatggtcccgccgttgtcctggttgtgacccgaccgggacgccatggagagactggtgtcgaagaaccagtcggtcccactggccctcgtccgccccaacctggtctacatggtcaccggaaatcctgcctctgatgagatcaagaggctgcctggagacatccaggtggtgcccattggagtgggccctaatggggttggaccagatgtaccagtggcctttaggacggagactactctagttctccgacggacctctgtaggtccaccacgggtaacctcacccgggattacccaacgtgcaggagctggagaggattggctggcccaatgcccctatcctcatccaggactttgagacgctcccccgagaggctcctgacctggtgctgcaggttgcacgtcctcgacctctcctaaccgaccgggttacggggataggagtaggtcctgaaactctgcgagggggctctccgaggactggaccacgacgtgaggtgctgctccggagaggggctgcagatccccaccctctcccctgcacctgactgcagccagcccctggacgtgatccttctcctggatggctcctccctccacgacgaggcctctccccgacgtctaggggtgggagaggggacgtggactgacgtcggtcggggacctgcactaggaagaggacctaccgaggaggagtttcccagcttcttattttgatgaaatgaagagtttcgccaaggctttcatttcaaaagccaatatagggcctcgtctcactcaggtgtcagtgctgctcaaagggtcgaagaataaaactactttacttctcaaagcggttccgaaagtaaagttttcggttatatcccggagcagagtgagtccacagtcacgacgagtatggaagcatcaccaccattgacgtgccatggaacgtggtcccggagaaagcccatttgctgagccttgtggacgtcatgcagcgggagggaggccctcataccttcgtagtggtggtaactgcacggtaccttgcaccagggcctctttcgggtaaacgactcggaacacctgcagtacgtcgccctccctccgggcagccaaatcggggatgccttgggctttgctgtgcgatacttgacttcagaaatgcatggtgccaggccgggagcctcaaaggcggtggtcatcctggtcgtcggtttagcccctacggaacccgaaacgacacgctatgaactgaagtctttacgtaccacggtccggccctcggagtttccgccaccagtaggaccagacggacgtctctgtggattcagtggatgcagcagctgatgccgccaggtccaacagagtgacagtgttccctattggaattggagatcgctacgatgcagtgcctgcagagacacctaagtcacctacgtcgtcgactacggcggtccaggttgtctcactgtcacaagggataaccttaacctctagcgatgctacgtccccagctacggatcttggcaggcccagcaggcgactccaacgtggtgaagctccagcgaatcgaagacctccctaccatggtcaccttgggcaattccttgggtcgatgcctagaaccgtccgggtcgtccgctgaggttgcaccacttcgaggtcgcttagcttctggagggatggtaccagtggaacccgttaaggaacctccacaaactgtgctctggatttgttaggatttgcatggatgaggatgggaatgagaagaggcccggggacgtctggaccttgccagaccagtgccacggaggtgtttgacacgagacctaaacaatcctaaacgtacctactcctacccttactcttctccgggcccctgcagacctggaacggtctggtcacggtgaccgtgacttgccagccagatggccagaccttgctgaagagtcatcgggtcaactgtgaccgggggctgaggccttcgtgccctaacagccagtcccctgtggcactgaacggtcggtctaccggtctggaacgacttctcagtagcccagttgacactggcccccgactccggaagcacgggattgtcggtcaggggacttaaagtggaagagacctgtggctgccgctggacctgcccctgygtgtgcacaggcagctccactcggcacatcgtgacctttgatgggcagaatttcaaaatttcaccttctctggacaccgacggcgacctggacggggacrcacacgtgtccgtcgaggtgagccgtgtagcactggaaactacccgtcttaaagttgctgactggcagctgttcttatgtcctatttcaaaacaaggagcaggacctggaggtgattctccataatggtgcctgcagccctggagcaaggcagggccgactgaccgtcgacaagaatacaggataaagttttgttcctcgtcctggacctccactaagaggtattaccacggacgtcgggacctcgttccgtcccgtgcatgaaatccatcgaggtgaagcacagtgccctctccgtcgagstgcacagtgacatggaggtgacggtgaatgggagactggtctctgttccttacgacgtactttaggtagctccacttcgtgtcacgggagaggcagctcsacgtgtcactgtacctccactgccacttaccctctgaccagagacaaggaatgctgggtgggaacatggaagtcaacgtttatggtgccatcatgcatgaggtcagattcaatcaccttggtcacatcttcacattcactccacaaaacaatgaacccacccttgtaccttcagttgcaaataccacggtagtacgtactccagtctaagttagtggaaccagtgtagaagtgtaagtgaggtgttttgttactgttccaactgcagctcagccccaagacttttgcttcaaagacgtatggtctgtgtgggatctgtgatgagaacggagccaatgacttcatgctgagggatcaaggttgacgtcgagtcggggttctgaaaacgaagtttctgcataccagacacaccctagacactactcttgcctcggttactgaagtacgactccctaggcacagtcaccacagactggaaaacacttgttcaggaatggactgtgcagcggccagggcagacgtgccagcccatcctggaggagcagtgtcttgtccccgtgtcagtggtgtctgaccttttgtgaacaagtccttacctgacacgtcgccggtcccgtctgcacggtcgggtaggacctcctcgtcacagaacaggccgacagctcccactgccaggtcctcctcttaccactgtttgctgaatgccacaaggtcctggctccagccacattctatgccatctgccagcaggacagggctgtcgagggtgacggtccaggaggagaatggtgacaaacgacttacggtgttccaggaccgaggtcggtgtaagatacggtagacggtcgtcctgtcttgccaccaggagcaagtgtgtgaggtgatcgcctcttatgcccacctctgtcggaccaacggggtctgcgttgactggaggacacctgatttctgtgctaacggtggtcctcgttcacacactccactagcggagaatacgggtggagacagcctggttgccccagacgcaactgacctcctgtggactaaagacacgaatgtcatgcccaccatctctggtctacaaccactgtgagcatggctgtccccggcactgtgatggcaacgtgagctcctgtggggaccatccctccgaagtacagtacgggtggtagagaccagatgttggtgacactcgtaccgacaggggccgtgacactaccgttgcactcgaggacacccctggtagggaggcttcgctgtttctgccctccagataaagtcatgttggaaggcagctgtgtccctgaagaggcctgcactcagtgcattggtgaggatggagtccagcaccagttcgacaaagacgggaggtctatttcagtacaaccttccgtcgacacagggacttctccggacgtgagtcacgtaaccactcctacctcaggtcgtggtcaacctggaagcctgggtcccggaccaccagccctgtcagatctgcacatgcctcagcgggcggaaggtcaactgcacaacgcagccctgccccacggccaaaggaccttcggacccagggcctggtggtcgggacagtctagacgtgtacggagtcgcccgccttccagttgacgtgttgcgtcgggacggggtgccggtttgctcccacgtgtggcctgtgtgaagtagcccgcctccgccagaatgcagaccagtgctgccccgagtatgagtgtgtgtgtgacccagtgagctgtgacccgagggtgcacaccggacacacttcatcgggcggaggcggtcttacgtctggtcacgacggggctcatactcacacacacactgggtcactcgacactggtgcccccagtgcctcactgtgaacgtggcctccagcccacactgaccaaccctggcgagtgcagacccaacttcacctgcgcctgcaggaaggaggagtgacgggggtcacggagtgacacttgcaccggaggtcgggtgtgactggttgggaccgctcacgtctgggttgaagtggacgcggacgtccttcctcctcaccaaaagagtgtccccaccctcctgccccccgcaccgtttgcccacccttcggaagacccagtgctgtgatgagtatgagtgtgcctgcaactgtgtcaacgttttctcacaggggtgggaggacggggggcgtggcaaacgggtgggaagccttctgggtcacgacactactcatactcacacggacgttgacacagttgtccacagtgagctgtccccttgggtacttggcctcaaccgccaccaatgactgtggctgtaccacaaccacctgccttcccgacaaggtgtgtgtccaccaggtgtcactcgacaggggaacccatgaaccggagttggcggtggttactgacaccgacatggtgttggtggacggaagggctgttccacacacaggtgggaagcaccatctaccctgtgggccagttctgggaggagggctgcgatgtgtgcacctgcaccgacatggaggatgccgtgatgggcctccgcgtggcccacttcgtggtagatgggacacccggtcaagaccctcctcccgacgctacacacgtggacgtggctgtacctcctacggcactacccggaggcgcaccgggtgtgctcccagaagccctgtgaggacagctgtcggtcgggcttcacttacgttctgcatgaaggcgagtgctgtggaaggtgcctgccatctgcctgtgagcacgagggtcttcgggacactcctgtcgacagccagcccgaagtgaatgcaagacgtacttccgctcacgacaccttccacggacggtagacggacactcgtggtgactggctcaccgcggggggactcccagtcttcctggaagagtgtcggctcccagtgggcctccccggagaacccctgcctcatcaatgagtgtgcaccactgaccgagtggcgcccccctgagggtcagaaggaccttctcacagccgagggtcacccggaggggcctcttggggacggagtagttactcacactccgagtgaaggaggaggtctttatacaacaaaggaacgtctcctgcccccagctggaggtccctgtctgcccctcgggctttcagctgagctgtaagacaggctcacttcctcctccagaaatatgttgtttccttgcagaggacgggggtcgacctccagggacagacggggagcccgaaagtcgactcgacattctgctcagcgtgctgcccaagctgtcgctgtgagcgcatggaggcctgcatgctcaatggcactgtcattgggcccgggaagactgtgatgatcgatgtgtgcgagtcgcacgacgggttcgacagcgacactcgcgtacctccggacgtacgagttaccgtgacagtaacccgggcccttctgacactactagctacacacgacgacctgccgctgcatggtgcaggtgggggtcatctctggattcaagctggagtgcaggaagaccacctgcaacccctgccccctgggttacaaggaagtgctggacggcgacgtaccacgtccacccccagtagagacctaagttcgacctcacgtccttctggtggacgttggggacgggggacccaatgttccttcaaaataacacaggtgaatgttgtgggagatgtttgcctacggcttgcaccattcagctaagaggaggacagatcatgacactgaagcgtgatgagacgctttttattgtgtccacttacaacaccctctacaaacggatgccgaacgtggtaagtcgattctcctcctgtctagtactgtgacttcgcactactctgcgaccaggatggctgtgatactcacttctgcaaggtcaatgagagaggagagtacttctgggagaagagggtcacaggctgcccaccctttgatgaacacaagggtcctaccgacactatgagtgaagacgttccagttactctctcctctcatgaagaccctcttctcccagtgtccgacgggtgggaaactacttgtgttctgtcttgctgagggaggtaaaattatgaaaattccaggcacctgctgtgacacatgtgaggagcctgagtgcaacgacatcactgccaggctgcagtatgacagaacgactccctccattttaatacttttaaggtccgtggacgacactgtgtacactcctcggactcacgttgctgtagtgacggtccgacgtcatactcaaggtgggaagctgtaagtctgaagtagaggtggatatccactactgccagggcaaatgtgccagcaaagccatgtactccattgacatcaacgatgtagttccacccttcgacattcagacttcatctccacctataggtgatgacggtcccgtttacacggtcgtttcggtacatgaggtaactgtagttgctacagcaggaccagtgctcctgctgctctccgacacggacggagcccatgcaggtggccctgcactgcaccaatggctctgttgtgtaccatgaggttctcaatcgtcctggtcacgaggacgacgagaggctgtgcctgcctcgggtacgtccaccgggacgtgacgtggttaccgagacaacacatggtactccaagagttagccatggagtgcaaatgctcccccaggaagtgcagcaagtga

SEQ ID NO: 28 - protein, 2813 aa, Homo sapiens
  VARIANT 2016: note = Xaa can be any naturally occurring amino acid
MIPARFAGVLLALALILPGTLCAEGTRGRSSTARCSLFGSDFVNTFDGSMYSFAGYCSYLLAGGCQKRSFSIIGDFQNGKRVSLSVYLGEFFDIHLFVNGTVTQGDQRVSMPYASKGLYLETEAGYYKLSGEAYGFVARIDGSGNFQVLLSDRYFNKTCGLCGNFNIFAEDDFMTQEGTLTSDPYDFANSWALSSGEQWCERASPPSSSCNISSGEMQKGLWEQCQLLKSTSVFARCHPLVDPEPFVALCEKTLCECAGGLECACPALLEYARTCAQEGMVLYGWTDHSACSPVCPAGMEYRQCVSPCARTCQSLHINEMCQERCVDGCSCPEGQLLDEGLCVESTECPCVHSGKRYPPGTSLSRDCNTCICRNSQWICSNEECPGECLVTGQSHFKSFDNRYFTFSGICQYLLARDCQDHSFSIVIETVQCADDRDAVCTRSVTVRLPGLHNSLVKLKHGAGVAMDGQDIQLPLLKGDLRIQHTVTASVRLSYGEDLQMDWDGRGRLLVKLSPVYAGKTCGLCGNYNGNQGDDFLTPSGLAEPRVEDFGNAWKLHGDCQDLQKQHSDPCALNPRMTRFSEEACAVLTSPTFEACHRAVSPLPYLRNCRYDVCSCSDGRECLCGALASYAAACAGRGVRVAWREPGRCELNCPKGQVYLQCGTPCNLTCRSLSYPDEECNEACLEGCFCPPGLYMDERGDCVPKAQCPCYYDGEIFQPEDIFSDHHTMCYCEDGFMHCTMSGVPGSLLPDAVLSSPLSHRSKRSLSCRPPMVKLVCPADNLRAEGLECTKTCQNYDLECMSMGCVSGCLCPPGMVRHENRCVALERCPCFHQGKEYAPGETVKIGCNTCVCRDRKWNCTDHVCDATCSTIGMAHYLTFDGLKYLFPGECQYVLVQDYCGSNPGTFRILVGNKGCSHPSVKCKKRVTILVEGGEIELFDGEVNVKRPMKDETHFEVVESGRYIILLLGKALSVVWDRHLSISVVLKQTYQEKVCGLCGNFDGIQNNDLTSSNLQVEEDPVDFGNSWKVSSQCADTRKVPLDSSPATCHNNIMKQTMVDSSCRILTSDVFQDCNKLVDPEPYLDVCIYDTCSCESIGDCACFCDTIAAYAHVCAQHGKVVTWRTATLCPQSCEERNLRENGYECEWRYNSCAPACQVTCQHPEPLACPVQCVEGCHAHCPPGKILDELLQTCVDPEDCPVCEVAGRRFASGKKVTLNPSDPEHCQICHCDVVNLTCEACQEPGGLVVPPTDAPVSPTTLYVEDISEPPLHDFYCSRLLDLVFLLDGSSRLSEAEFEVLKAFVVDMMERLRISQKWVRVAVVEYHDGSHAYIGLKDRKRPSELRRIASQVKYAGSQVASTSEVLKYTLFQIFSKIDRPEASRIALLLMASQEPQRMSRNFVRYVQGLKKKKVIVIPVGIGPHANLKQIRLIEKQAPENKAFVLSSVDELEQQRDEIVSYLCDLAPEAPPPTLPPDMAQVTVGPGLLGVSTLGPKRNSMVLDVAFVLEGSDKIGEADFNRSKEFMEEVIQRMDVGQDSIHVTVLQYSYMVTVEYPFSEAQSKGDILQRVREIRYQGGNRTNTGLALRYLSDHSFLVSQGDREQAPNLVYMVTGNPASDEIKRLPGDIQVVPIGVGPNANVQELERIGWPNAPILIQDFETLPREAPDLVLQRCCSGEGLQIPTLSPAPDCSQPLDVILLLDGSSSFPASYFDEMKSFAKAFISKANIGPRLTQVSVLQYGSITTIDVPWNVVPEKAHLLSLVDVMQREGGPSQIGDALGFAVRYLTSEMHGARPGASKAVVILVTDVSVDSVDAAADAARSNRVTVFPIGIGDRYDAAQLRILAGPAGDSNVVKLQRIEDLPTMVTLGNSFLHKLCSGFVRICMDEDGNEKRPGDVWTLPDQCHTVTCQPDGQTLLKSHRVNCDRGLRPSCPNSQSPVKVEETCGCRWTCPCVCTGSSTRHIVTFDGQNFKLTGSCSYVLFQNKEQDLEVILHNGACSPGARQGCMKSIEVKHSALSVEXHSDMEVTVNGRLVSVPYVGGNMEVNVYGAIMHEVRFNHLGHIFTFTPQNNEFQLQLSPKTFASKTYGLCGICDENGANDFMLRDGTVTTDWKTLVQEWTVQRPGQTCQPILEEQCLVPDSSHCQVLLLPLFAECHKVLAPATFYAICQQDSCHQEQVCEVIASYAHLCRTNGVCVDWRTPDFCAMSCPPSLVYNHCEHGCPRHCDGNVSSCGDHPSEGCFCPPDKVMLEGSCVPEEACTQCIGEDGVQHQFLEAWVPDHQPCQICTCLSGRKVNCTTQPCPTAKAPTCGLCEVARLRQNADQCCPEYECVCDPVSCDLPPVPHCERGLQPTLTNPGECRPNFTCACRKEECKRVSPPSCPPHRLPTLRKTQCCDEYECACNCVNSTVSCPLGYLASTATNDCGCTTTTCLPDKVCVHRSTIYPVGQFWEEGCDVCTCTDMEDAVMGLRVAQCSQKPCEDSCRSGFTYVLHEGECCGRCLPSACEVVTGSPRGDSQSSWKSVGSQWASPENPCLINECVRVKEEVFIQQRNVSCPQLEVPVCPSGFQLSCKTSACCPSCRCERMEACMLNGTVIGPGKTVMIDVCTTCRCMVQVGVISGFKLECRKTTCNPCPLGYKEENNTGECCGRCLPTACTIQLRGGQIMTLKRDETLQDGCDTHFCKVNERGEYFWEKRVTGCPPFDEHKCLAEGGKIMKIPGTCCDTCEEPECNDITARLQYVKVGSCKSEVEVDIHYCQGKCASKAMYSIDINDVQDQCSCCSPTRTEPMQVALHCTNGSVVYHEVLNAMECKCSPRKCSK

SEQ ID NO: 29 - protein, 4 aa, synthetic construct
  REGION 1..4: note = human IgG1
ELLG

SEQ ID NO: 30 - protein, 42 aa, synthetic construct
  REGION 1..42: note = XTEN AE42-4
GAPGSPAGSPTSTEEGTSESATPESGPGSEPATSGSETPASS

SEQ ID NO: 31 - DNA, 126 bp, synthetic construct
  misc_feature 1..126: note = XTEN AE42-4
  source 1..126: mol_type = other DNA
ggcgcgccaggttctcctgctggctcccccacctcaacagaagaggggacaagcgaaagcgctacgcctgagagtggccctggctctgagccagccacctccggctctgaaacccctgcctcgagc

SEQ ID NO: 32 - protein, 144 aa, synthetic construct
  REGION 1..144: note = XTEN AE144-2A
TSTEPSEGSAPGSPAGSPTSTEEGTSTEPSEGSAPGTSTEPSEGSAPGTSESATPESGPGTSTEPSEGSAPGTSESATPESGPGSEPATSGSETPGTSTEPSEGSAPGTSTEPSEGSAPGTSESATPESGPGTSESATPESGPG

SEQ ID NO: 33 - DNA, 450 bp, synthetic construct
  misc_feature 1..450: note = XTEN AE144-2A
  source 1..450: mol_type = other DNA
ggcgcgccaaccagtacggagccgtccgaggggagcgcaccaggaagcccggctgggagcccgacttctaccgaagagggtacatctaccgaaccaagtgaaggttcagcaccaggcacctcaacagaaccctctgagggctcggcgcctggtacaagtgagtccgccaccccagaatccgggcctgggacaagcacagaaccttcggaagggagtgcccctggaacatccgaatcggcaaccccagaatcagggccaggatctgagcccgcgacttcgggctccgagacgcctgggacatccaccgagccctccgaaggatcagccccaggcaccagcacggagccctctgagggaagcgcacctggtaccagcgaaagcgcaactcccgaatcaggtcccggtacgagcgagtcggcgaccccggagagcgggccaggtgcctcgagc

SEQ ID NO: 34 - protein, 144 aa, synthetic construct
  REGION 1..144: note = XTEN AE144-3B
SPAGSPTSTEEGTSESATPESGPGSEPATSGSETPGTSESATPESGPGTSTEPSEGSAPGTSTEPSEGSAPGTSTEPSEGSAPGTSTEPSEGSAPGTSTEPSEGSAPGTSTEPSEGSAPGSPAGSPTSTEEGTSTEPSEGSAPG

SEQ ID NO: 35 - DNA, 450 bp, synthetic construct
  misc_feature 1..450: note = XTEN AE144-3B
  source 1..450: mol_type = other DNA
ggcgcgccaagtcccgctggaagcccaactagcaccgaagaggggacctcagagtccgccacccccgagtccggccctggctctgagcctgccactagcggctccgagactcctggcacatccgaaagcgctacacccgagagtggacccggcacctctaccgagcccagtgagggctccgcccctggaacaagcaccgagcccagcgaaggcagcgccccagggacctccacagagcccagtgaaggcagtgctcctggcaccagcaccgaaccaagcgagggctctgcacccgggacctccaccgagccaagcgaaggctctgcccctggcacttccaccgagcccagcgaaggcagcgcccctgggagccccgctggctctcccaccagcactgaggagggcacatctaccgaaccaagtgaaggctctgcaccaggtgcctcgagc

SEQ ID NO: 36 - protein, 144 aa, synthetic construct
  REGION 1..144: note = XTEN AE144-4A
TSESATPESGPGSEPATSGSETPGTSESATPESGPGSEPATSGSETPGTSESATPESGPGTSTEPSEGSAPGTSESATPESGPGSPAGSPTSTEEGSPAGSPTSTEEGSPAGSPTSTEEGTSESATPESGPGTSTEPSEGSAPG

SEQ ID NO: 37 - DNA, 450 bp, synthetic construct
  misc_feature 1..450: note = XTEN AE144-4A
  source 1..450: mol_type = other DNA
ggcgcgccaacgtccgaaagtgctacccctgagtcaggccctggtagtgagcctgccacaagcggaagcgaaactccggggacctcagagtctgccactcccgaatcggggccaggctctgaaccggccacttcagggagcgaaacaccaggaacatcggagagcgctaccccggagagcgggccaggaactagtactgagcctagcgagggaagtgcacctggtacaagcgagtccgccacacccgagtctggccctggctctccagcgggctcacccacgagcactgaagagggctctcccgctggcagcccaacgtcgacagaagaaggatcaccagcaggctcccccacatcaacagaggagggtacatcagaatctgctactcccgagagtggacccggtacctccactgagcccagcgaggggagtgcaccaggtgcctcgagc

SEQ ID NO: 38 - protein, 144 aa, synthetic construct
  REGION 1..144: note = XTEN AE144-5A
TSESATPESGPGSEPATSGSETPGTSESATPESGPGSEPATSGSETPGTSESATPESGPGTSTEPSEGSAPGSPAGSPTSTEEGTSESATPESGPGSEPATSGSETPGTSESATPESGPGSPAGSPTSTEEGSPAGSPTSTEEG

SEQ ID NO: 39 - DNA, 450 bp, synthetic construct
  misc_feature 1..450: note = XTEN AE144-5A
  source 1..450: mol_type = other DNA
ggcgcgccaacatcagagagcgccacccctgaaagtggtcccgggagcgagccagccacatctgggtcggaaacgccaggcacaagtgagtctgcaactcccgagtccggacctggctccgagcctgccactagcggctccgagactccgggaacttccgagagcgctacaccagaaagcggacccggaaccagtaccgaacctagcgagggctctgctccgggcagcccagccggctctcctacatccacggaggagggcacttccgaatccgccaccccggagtcagggccaggatctgaacccgctacctcaggcagtgagacgccaggaacgagcgagtccgctacaccggagagtgggccagggagccctgctggatctcctacgtccactgaggaagggtcaccagcgggctcgcccaccagcactgaagaaggtgcctcgagc

SEQ ID NO: 40 - protein, 144 aa, synthetic construct
  REGION 1..144: note = XTEN AE144-6B
TSTEPSEGSAPGTSESATPESGPGTSESATPESGPGTSESATPESGPGSEPATSGSETPGSEPATSGSETPGSPAGSPTSTEEGTSTEPSEGSAPGTSTEPSEGSAPGSEPATSGSETPGTSESATPESGPGTSTEPSEGSAPG

SEQ ID NO: 41 - DNA, 450 bp, synthetic construct
  misc_feature 1..450: note = XTEN AE144-6B
  source 1..450: mol_type = other DNA
ggcgcgccaacatctaccgagccttccgaaggctctgcccctgggacctcagaatctgcaacccctgaaagcggccctggaacctccgaaagtgccactcccgagagcggcccagggacaagcgagtcagcaacccctgagtctggacccggcagcgagcctgcaacctctggctcagagactcccggctcagaacccgctacctcaggctccgagacacccggctctcctgctgggagtcccacttccaccgaggaaggaacatccactgagcctagtgagggctctgcccctggaaccagcacagagccaagtgagggcagtgcaccaggatccgagccagcaaccagcgggtccgagactcccgggacctctgagtctgccaccccagagagcggacccggcacttcaaccgagccctccgaaggatcagcaccaggtgcctcgagc

SEQ ID NO: 42 - protein, 144 aa, synthetic construct
  REGION 1..144: note = XTEN AG144-1
PGSSPSASTGTGPGSSPSASTGTGPGTPGSGTASSSPGSSTPSGATGSPGSSPSASTGTGPGASPGTSSTGSPGTPGSGTASSSPGSSTPSGATGSPGTPGSGTASSSPGASPGTSSTGSPGASPGTSSTGSPGTPGSGTASSS

SEQ ID NO: 43 - DNA, 450 bp, synthetic construct
  misc_feature 1..450: note = XTEN AG144-1
  source 1..450: mol_type = other DNA
ggcgcgccacccgggtcgtccccgtcggcgtccaccggaacagggccagggtcatccccgtcagcgtcgactgggacgggacccgggacacccggttcggggactgcatcctcctcgcctggttcgtccaccccgtcaggagccacgggttcgccgggaagcagcccaagcgcatccactggtacagggcctggggcttcaccgggtacttcatccacggggtcaccgggaacgcccggatcggggacggcttcctcatcaccaggatcgtcaacaccctcgggcgcaacgggcagccccggaacccctggttcgggtacggcgtcgtcgagccccggtgcgagcccgggaacaagctcgacaggatcgcctggggcgtcacccggcacgtcgagcacaggcagccccggaacccctggatcgggaaccgcgtcgtcaagcgcctcgagc

SEQ ID NO: 44 - protein, 144 aa, synthetic construct
  REGION 1..144: note = XTEN AG144-A
GASPGTSSTGSPGSSPSASTGTGPGSSPSASTGTGPGTPGSGTASSSPGSSTPSGATGSPGSSPSASTGTGPGASPGTSSTGSPGTPGSGTASSSPGSSTPSGATGSPGTPGSGTASSSPGASPGTSSTGSPGASPGTSSTGSP

SEQ ID NO: 45 - DNA, 450 bp, synthetic construct
  misc_feature 1..450: note = XTEN AG144-A
  source 1..450: mol_type = other DNA
ggcgcgccaggtgcctcgccgggaacatcatcaactggttcacccgggtcatccccctcggcctcaaccgggacgggtcccggctcatcccccagcgccagcactggaacaggtcctggcactcctggttccggtacggcatcgtcatccccgggaagctcaacaccgtccggagcgacaggatcacctggctcgtcaccttcggcgtcaactggaacggggccaggggcctcacccggaacgtcctcgactgggtcgcctggtacgccgggatcaggaacggcctcatcctcgcctgggtcctcaacgccctcgggtgcgactggttcgccgggaactcctggctcggggacggcctcgtcgtcgcctggggcatcaccggggacgagctccacggggtcccctggagcgtcaccggggacctcctcgacaggtagcccggcctcgagc

SEQ ID NO: 46 - protein, 144 aa, synthetic construct
  REGION 1..144: note = XTEN AG144-B
GTPGSGTASSSPGSSTPSGATGSPGASPGTSSTGSPGTPGSGTASSSPGSSTPSGATGSPGSSPSASTGTGPGSSPSASTGTGPGSSTPSGATGSPGSSTPSGATGSPGASPGTSSTGSPGASPGTSSTGSPGASPGTSSTGSP

SEQ ID NO: 47 - DNA, 450 bp, synthetic construct
  misc_feature 1..450: note = XTEN AG144-B
  source 1..450: mol_type = other DNA
ggcgcgccaggtacaccgggcagcggcacggcttcgtcgtcacccggctcgtccacaccgtcgggagctacgggaagcccaggagcgtcaccgggaacgtcgtcaacggggtcaccgggtacgccaggtagcggcacggccagcagctcgccaggttcatcgaccccgtcgggagcgactgggtcgcccggatcaagcccgtcagcttccactggaacaggacccgggtcgtcgccgtcagcctcaacggggacaggacctggttcatcgacgccgtcaggggcgacaggctcgcccggatcgtcaacaccctcgggggcaacggggagccctggtgcgtcgcctggaacctcatccaccggaagcccgggggcctcgccgggtacgagctccacgggatcgcccggagcgtcccccggaacttcaagcacagggagccctgcctcgagc

SEQ ID NO: 48 - protein, 144 aa, synthetic construct
  REGION 1..144: note = XTEN AG144-C
GTPGSGTASSSPGASPGTSSTGSPGASPGTSSTGSPGASPGTSSTGSPGSSPSASTGTGPGTPGSGTASSSPGASPGTSSTGSPGASPGTSSTGSPGASPGTSSTGSPGSSTPSGATGSPGSSTPSGATGSPGASPGTSSTGSP

SEQ ID NO: 49 - DNA, 450 bp, synthetic construct
  misc_feature 1..450: note = XTEN AG144-C
  source 1..450: mol_type = other DNA
ggcgcgccaggtacacccggatcgggtacagcgtcatcgagccccggtgcgtcacctggtacgtcgagcacggggtcgccaggggcgtcccctgggacgtcctcaacaggctcgcccggtgcgtcacccggcacgtcgtccacgggttcacctggtagctccccttccgcgtccactggcaccgggcctggaactccggggagcggcacagcgagctcgtcgccgggagcatcgcctgggacatcgagcaccgggtcgccaggagcatcgcccggaacatccagcacaggaagccccggcgcgtcgcccgggacatcaagcacaggttccccgggatcgagcacgccgtccggagccactggatcaccagggagctcgacaccttccggcgcaacgggatcgcccggagccagcccgggtacgtcaagcactggctcccctgcctcgagc

SEQ ID NO: 50 - protein, 144 aa, synthetic construct
  REGION 1..144: note = XTEN AG144-F
GSSPSASTGTGPGSSPSASTGTGPGASPGTSSTGSPGASPGTSSTGSPGSSTPSGATGSPGSSPSASTGTGPGASPGTSSTGSPGSSPSASTGTGPGTPGSGTASSSPGSSTPSGATGSPGSSTPSGATGSPGASPGTSSTGSP

SEQ ID NO: 51 - DNA, 450 bp, synthetic construct
  misc_feature 1..450: note = XTEN AG144-F
  source 1..450: mol_type = other DNA
ggcgcgccaggctccagcccctccgcgagcacgggaaccggaccaggttcgtcaccctcagcatcaacggggacgggaccgggggcgtcaccaggaacgtcctccaccggctcgccgggtgcatcacccggaacgtcatcgaccggatcgccagggagctcgacgccatcaggcgcaacaggatcacctggctcaagccctagcgcgtcaaccggcacgggtccgggtgcctcccctggcacgtccagcaccggatcacccggatcgagcccatccgcctcaaccggaaccggacccggtacaccagggtcgggaacagcctcctcgtcaccaggctcctcaaccccctcgggagccacgggttcgcccggttcgtcaacgccttccggagcaactggtagccccggagcatcgccaggaacttcgagcacggggtcgcccgcctcgagc